European Patent Application EP 4 159 745 A1, published April 5, 2023. Title: A S100A8-inhibiting peptide and a drug for disease. Applicant: TOKYO WOMEN'S MEDICAL UNIVERSITY. The sequence listing filed with the application follows.

SEQUENCE LISTING (13 sequences)

SEQ ID NO: 1 - protein, 10 aa, Artificial Sequence
  Description of artificial sequence
FQEFAILVIK

SEQ ID NO: 2 - protein, 5 aa, Artificial Sequence
  Description of artificial sequence
ILVIK

SEQ ID NO: 3 - protein, 9 aa, Artificial Sequence
  Description of artificial sequence
FQEFAILVI

SEQ ID NO: 4 - protein, 7 aa, Artificial Sequence
  Description of artificial sequence
QEFAILV

SEQ ID NO: 5 - protein, 7 aa, Artificial Sequence
  Description of artificial sequence
EFAILVI

SEQ ID NO: 6 - protein, 6 aa, Artificial Sequence
  Description of artificial sequence
EFAILV

SEQ ID NO: 7 - protein, 6 aa, Artificial Sequence
  Description of artificial sequence
FAILVI

SEQ ID NO: 8 - protein, 5 aa, Artificial Sequence
  Description of artificial sequence
FAILV

SEQ ID NO: 9 - protein, 5 aa, Artificial Sequence
  Description of artificial sequence
AILVI

SEQ ID NO: 10 - protein, 6 aa, Artificial Sequence
  Description of artificial sequence
AILVIK

SEQ ID NO: 11 - protein, 8 aa, Artificial Sequence
  Description of artificial sequence
FQEFAILV

SEQ ID NO: 12 - protein, 8 aa, Artificial Sequence
  Description of artificial sequence
QEFAILVI

SEQ ID NO: 13 - protein, 10 aa, Artificial Sequence
  Description of artificial sequence
FQEFLILVIK